European Patent Specification EP 3 461 848 B1, published October 11, 2023. Title: Transgenic Mice. Applicant: Crescendo Biologics Limited. The sequence listing filed with the application follows.

SEQUENCE LISTING (147 sequences)

SEQ ID NO: 1 - DNA, 88 bp, Artificial Sequence
  Primer
gacattctgccattgtgattactactactactacggtatggacgtctgggggcaagggaccacggtcaccgtctcctcaggtaagaat

SEQ ID NO: 2 - DNA, 31 bp, Artificial Sequence
  Primer
ttgaggaccagagagggataaaagagaaatg

SEQ ID NO: 3 - DNA, 26 bp, Artificial Sequence
  Primer
agaggacgtatagggaggaggggttc

SEQ ID NO: 4 - DNA, 21 bp, Artificial Sequence
  Primer
aacaccttcagcgatgcagac

SEQ ID NO: 5 - DNA, 546 bp, Artificial Sequence
  Primer
tcatgcccctagagttggctgaagggccagatccacctactctagaggcatctctccctgtctgtgaaggcttccaaagtcacgttcctgtggctagaaggcagctccatagccctgctgcagtttcgtcctgtataccaggttcacctactaccatatctagccctgcctgccttaagagtagcaacaaggaaatagcagggtgtagagggatctcctgtctgacaggaggcaagaagacagattcttacccctccatttctcttttatccctctctggtcctcagaagaggacgtatagggaggaggggttcactagaggtgaggctcaagccattagcctgcctaaaccaaccaggctggacagccatcaccaggaaatggatctcagcccagaagatcgaaagttgttcttctcccttctggagatttctatgtcctttacactcattggttaatatcctgggttggattcccacacatcttgacaaacagagacaattgagtatcaccagccaaaagtcatacccaaaaacagcctggcat

SEQ ID NO: 6 - DNA, 57 bp, Artificial Sequence
  Primer
gaacccctcctccctatacgtcctctttgaggaccagagagggataaaagagaaatg

SEQ ID NO: 7 - DNA, 26 bp, Artificial Sequence
  Primer
agaggacgtatagggaggaggggttc

SEQ ID NO: 8 - DNA, 21 bp, Artificial Sequence
  Primer
atgccaggctgtttttgggta

SEQ ID NO: 9 - DNA, 80 bp, Artificial Sequence
  Primer
tacatcttttttcctctctgtctgcatcgctgaaggtgtttcgtcgccgcacttatgactgtcttctttatcatgcaact

SEQ ID NO: 10 - DNA, 626 bp, Artificial Sequence
  Primer
acggctcaggaggaaaaggcactctgtgtggagctcttcagtgggtatgaaatggtgatggagaagcccaggtgcactgaaaatccaggagctgaatttgatcaccaggacgcatatggtagagaggaaaatgaattgattcccaaatgttctcctctatgtgtgcaccgtggcatgtgcatgcacacaattacacataaacacattcaacataaatacaacacacatatacacgctgcacacacatacacacacagaacacacaccacacacacacaccacacacaatcacacacatattccacacagtacaccacaaacatctatacacaccacacacacacagacacacacacacacacattcatacacagcacaacacaaacatctatacacaacacacacacaatacacatagtcacacgcatattcactcacacacatattcacccacacacaatcatacatagacacattcaacataaacacaacaccacacacacacacacttgcacacacaaatgtaatgatttttttaaggactacatcttttttcctctctgtctgcatcgctgaaggtgttcaattgccaaaatcacaggtgagcccagatgcatacccgggac

SEQ ID NO: 11 - DNA, 22 bp, Artificial Sequence
  Primer
acggctcaggaggaaaaggcac

SEQ ID NO: 12 - DNA, 43 bp, Artificial Sequence
  Primer
tcacctgtgattttggcaattgaacaccttcagcgatgcagac

SEQ ID NO: 13 - DNA, 43 bp, Artificial Sequence
  Primer
gtcccgggtatgcatctgggctcacctgtgattttggcaattg

SEQ ID NO: 14 - DNA, 766 bp, Artificial Sequence
  Primer
gaggtacagggggctcatgggtttataagttcaggtttataccaaggtttcggggggtagcctgaggctcatgtaccttcttgtggtagcccccaggttctgtgcatggtactgctcagttactggcatggcttctgggaaggctgggctcccacgtcccctgtggacacatggttacgccaagaacagaactacaaagttaggagttaccattcccacctgcacctgtatctccagtacctgggtttctaagacgtagtgagtcctcttgccaaccagggtctgccacaatggtcaggcacagctgtgggccggtcagccccatcaggtcacaccagcaggtcccaggagcacagagcttaaatgccccctagtgtccctagtgaggctccggtgcccgtcagtgggcagagcgcacatcgcccacagtccccgagaagttggggggaggggtcggcaattgaaccggtgcctagagaaggtggcgcggggtaaactgggaaagtgatgtcgtgtactggctccgcctttttcccgagggtgggggagaaccgtatataagtgcagtagtcgccgtgaacgttctttttcgcaacgggtttgccgccagaacacaggtaagtgccgtgtgtggttcccgcgggcctggcctctttacgggttatggcccttgcgtgccttgaattacttccacctggctgcagtacgtgattcttgatcccgagcttcgggttggaagtgggtgggagagttcgaggccttgcgc

SEQ ID NO: 15 - DNA, 22 bp, Artificial Sequence
  Primer
gaggtacagggggctcatgggt

SEQ ID NO: 16 - DNA, 33 bp, Artificial Sequence
  Primer
agcctcactagggacactagggggcatttaagc

SEQ ID NO: 17 - DNA, 33 bp, Artificial Sequence
  Primer
ccctagtgtccctagtgaggctccggtgcccgt

SEQ ID NO: 18 - DNA, 20 bp, Artificial Sequence
  Primer
gcgcaaggcctcgaactctc

SEQ ID NO: 19 - DNA, 23 bp, Artificial Sequence
  Primer
ggttggattctatcttcgcatgg

SEQ ID NO: 20 - DNA, 23 bp, Artificial Sequence
  Primer
tgggtcctgtctttctacctttg

SEQ ID NO: 21 - DNA, 23 bp, Artificial Sequence
  Primer
gctccttgctgggtcttaatgtt

SEQ ID NO: 22 - DNA, 25 bp, Artificial Sequence
  Primer
ttagaaccgtgtcttctacaattga

SEQ ID NO: 23 - DNA, 20 bp, Artificial Sequence
  Primer
gggtaggaggttgttggtta

SEQ ID NO: 24 - DNA, 34 bp, Artificial Sequence
  Primer
cccgctgggctctgcaagagaggagaatgtgtga

SEQ ID NO: 25 - DNA, 31 bp, Artificial Sequence
  Primer
ctctcttgcagagcccagcgggcccatttca

SEQ ID NO: 26 - DNA, 23 bp, Artificial Sequence
  Primer
gcttgtttttatatcgagcttgc

SEQ ID NO: 27 - DNA, 22 bp, Artificial Sequence
  Primer
tcagtctcacttgcctggtcgt

SEQ ID NO: 28 - DNA, 22 bp, Artificial Sequence
  Primer
ctttgtagcacatgcgtcatcc

SEQ ID NO: 29 - DNA, 22 bp, Artificial Sequence
  Primer
tgaaggcatgaaggagttgagc

SEQ ID NO: 30 - DNA, 22 bp, Artificial Sequence
  Primer
acaaccccctatcctacacatt

SEQ ID NO: 31 - DNA, 20 bp, Artificial Sequence
  Primer
gggtcctggcaacattagcg

SEQ ID NO: 32 - DNA, 34 bp, Artificial Sequence
  Primer
cactctgggctctgcaagaaaggaggatgtgtga

SEQ ID NO: 33 - DNA, 32 bp, Artificial Sequence
  Primer
ctttcttgcagagcccagagtgcccataacac

SEQ ID NO: 34 - DNA, 22 bp, Artificial Sequence
  Primer
tggtgttcagcaggctaatttg

SEQ ID NO: 35 - DNA, 22 bp, Artificial Sequence
  Primer
caggccccacttctttacctaa

SEQ ID NO: 36 - DNA, 25 bp, Artificial Sequence
  Primer
ttgttagttcatcacagggcaattc

SEQ ID NO: 37 - DNA, 27 bp, Artificial Sequence
  Primer
agagccccctgtctgataagaatctgg

SEQ ID NO: 38 - DNA, 22 bp, Artificial Sequence
  Primer
gagtccccatccccaaggctgg

SEQ ID NO: 39 - DNA, 32 bp, Artificial Sequence
  Primer
gatggtgaaggttaggatgtctgtggagggac

SEQ ID NO: 40 - DNA, 24 bp, Artificial Sequence
  Primer
ccatcttcccaccatccagtgagc

SEQ ID NO: 41 - DNA, 24 bp, Artificial Sequence
  Primer
gcaacagtggtaggtcgcttgtgg

SEQ ID NO: 42 - DNA, 24 bp, Artificial Sequence
  Primer
ggagatcaggaatgagggacaaac

SEQ ID NO: 43 - DNA, 21 bp, Artificial Sequence
  Primer
gcctttcccatgctcttgctg

SEQ ID NO: 44 - DNA, 22 bp, Artificial Sequence
  Primer
ggcaggaaagaagggttaagat

SEQ ID NO: 45 - DNA, 20 bp, Artificial Sequence
  Primer
gagggagcaccaatgagaag

SEQ ID NO: 46 - DNA, 20 bp, Artificial Sequence
  Primer
cagatgaggggaatgcaaat

SEQ ID NO: 47 - DNA, 30 bp, Artificial Sequence
  Primer
cccaagcttggtgcctctgatcccagggct

SEQ ID NO: 48 - DNA, 27 bp, Artificial Sequence
  Primer
gctctagatctgggctcacactcacct

SEQ ID NO: 49 - DNA, 30 bp, Artificial Sequence
  Primer
cccaagcttgaagccagtcaagggggcttc

SEQ ID NO: 50 - DNA, 27 bp, Artificial Sequence
  Primer
gctctagaggggttttcacactgtgtc

SEQ ID NO: 51 - DNA, 30 bp, Artificial Sequence
  Primer
cccaagcttgagtccagtccagggagatct

SEQ ID NO: 52 - DNA, 27 bp, Artificial Sequence
  Primer
gctctagaggggttttcacactgtgtc

SEQ ID NO: 53 - DNA, 28 bp, Artificial Sequence
  Primer
cccaagctttcacagcagcattcacaga

SEQ ID NO: 54 - DNA, 26 bp, Artificial Sequence
  Primer
ggaattcctgacttcccctcactgtg

SEQ ID NO: 55 - DNA, 20 bp, Artificial Sequence
  Primer
ggggctggagggagtaatag

SEQ ID NO: 56 - DNA, 20 bp, Artificial Sequence
  Primer
acttagctcggaccacagga

SEQ ID NO: 57 - DNA, 20 bp, Artificial Sequence
  Primer
atgatggagtttgggctgag

SEQ ID NO: 58 - DNA, 20 bp, Artificial Sequence
  Primer
ggaaatcagccttcatctgc

SEQ ID NO: 59 - DNA, 20 bp, Artificial Sequence
  Primer
gggtactgccttctcgtcag

SEQ ID NO: 60 - DNA, 20 bp, Artificial Sequence
  Primer
atttgcagataggcgatgct

SEQ ID NO: 61 - DNA, 20 bp, Artificial Sequence
  Primer
ccacgctggtcagttttgta

SEQ ID NO: 62 - DNA, 20 bp, Artificial Sequence
  Primer
gctgggaataggggactctc

SEQ ID NO: 63 - DNA, 20 bp, Artificial Sequence
  Primer
ggggtgagacacctgaagaa

SEQ ID NO: 64 - DNA, 20 bp, Artificial Sequence
  Primer
gagtgcaggaaaatcatcca

SEQ ID NO: 65 - DNA, 20 bp, Artificial Sequence
  Primer
gcacaggtttgtggcattta

SEQ ID NO: 66 - DNA, 20 bp, Artificial Sequence
  Primer
tgcagcggtaggttttcttt

SEQ ID NO: 67 - DNA, 20 bp, Artificial Sequence
  Primer
gcccttcacagagtccacat

SEQ ID NO: 68 - DNA, 20 bp, Artificial Sequence
  Primer
actccaaggcctttccactt

SEQ ID NO: 69 - DNA, 20 bp, Artificial Sequence
  Primer
atctcttcccctgcacttcc

SEQ ID NO: 70 - DNA, 20 bp, Artificial Sequence
  Primer
ctaccaaacgacccagcaat

SEQ ID NO: 71 - DNA, 20 bp, Artificial Sequence
  Primer
ccatcctcagcaacatctga

SEQ ID NO: 72 - DNA, 20 bp, Artificial Sequence
  Primer
gcatgaaaggtcctgctacc

SEQ ID NO: 73 - DNA, 20 bp, Artificial Sequence
  Primer
gggtggagagaccagtgtgt

SEQ ID NO: 74 - DNA, 20 bp, Artificial Sequence
  Primer
ttaggtgctgggagctcatt

SEQ ID NO: 75 - DNA, 20 bp, Artificial Sequence
  Primer
aggaccatggacaagagtgc

SEQ ID NO: 76 - DNA, 20 bp, Artificial Sequence
  Primer
ttggaaggatgggctgtatc

SEQ ID NO: 77 - DNA, 20 bp, Artificial Sequence
  Primer
gggagaatcccctagagcac

SEQ ID NO: 78 - DNA, 20 bp, Artificial Sequence
  Primer
gtggatgtcgatgcaaaatg

SEQ ID NO: 79 - DNA, 20 bp, Artificial Sequence
  Primer
agctccatgtaggctgtgct

SEQ ID NO: 80 - DNA, 20 bp, Artificial Sequence
  Primer
atggactggacctggaggat

SEQ ID NO: 81 - DNA, 20 bp, Artificial Sequence
  Primer
ggagttcttggcgttgtctc

SEQ ID NO: 82 - DNA, 20 bp, Artificial Sequence
  Primer
aggactcaccatggagttgg

SEQ ID NO: 83 - DNA, 20 bp, Artificial Sequence
  Primer
ctcaggctgttcatttgcag

SEQ ID NO: 84 - DNA, 20 bp, Artificial Sequence
  Primer
gagctgggttttccttgttg

SEQ ID NO: 85 - DNA, 20 bp, Artificial Sequence
  Primer
ggcattttctctggagatgg

SEQ ID NO: 86 - DNA, 20 bp, Artificial Sequence
  Primer
aggactcaccatggagttgg

SEQ ID NO: 87 - DNA, 20 bp, Artificial Sequence
  Primer
gagtcatcagggtcggtgtc

SEQ ID NO: 88 - DNA, 20 bp, Artificial Sequence
  Primer
acgaccaccgtgagaaaaac

SEQ ID NO: 89 - DNA, 20 bp, Artificial Sequence
  Primer
gctggtgggtgtgatgtatg

SEQ ID NO: 90 - DNA, 20 bp, Artificial Sequence
  Primer
cttcccttgaccgaagacag

SEQ ID NO: 91 - DNA, 20 bp, Artificial Sequence
  Primer
ctgtggtagccaccataccc

SEQ ID NO: 92 - DNA, 20 bp, Artificial Sequence
  Primer
tgggtagggacatagggaca

SEQ ID NO: 93 - DNA, 20 bp, Artificial Sequence
  Primer
gctcttgtgctcctggagag

SEQ ID NO: 94 - DNA, 20 bp, Artificial Sequence
  Primer
aaaaggtatccccaccttgc

SEQ ID NO: 95 - DNA, 20 bp, Artificial Sequence
  Primer
ggggagcatggtttttgtag

SEQ ID NO: 96 - DNA, 20 bp, Artificial Sequence
  Primer
ctgctgctgggaaaacaagt

SEQ ID NO: 97 - DNA, 20 bp, Artificial Sequence
  Primer
gcaggagagaggttgtgagg

SEQ ID NO: 98 - DNA, 20 bp, Artificial Sequence
  Primer
gctttccttctgcctccttt

SEQ ID NO: 99 - DNA, 20 bp, Artificial Sequence
  Primer
cctggtttgttcaggcatct

SEQ ID NO: 100 - DNA, 20 bp, Artificial Sequence
  Primer
cggagacagaaggtctctgg

SEQ ID NO: 101 - DNA, 20 bp, Artificial Sequence
  Primer
agccttttcagtttcggtca

SEQ ID NO: 102 - DNA, 21 bp, Artificial Sequence
  Primer
ctggtttccaagagaaaagga

SEQ ID NO: 103 - DNA, 24 bp, Artificial Sequence
  Primer
caagtgtacagtccccgaagcaag

SEQ ID NO: 104 - DNA, 22 bp, Artificial Sequence
  Primer
tgatacacgcaacacgcttgtc

SEQ ID NO: 105 - DNA, 22 bp, Artificial Sequence
  Primer
gaggtacagggggctcatgggt

SEQ ID NO: 106 - DNA, 25 bp, Artificial Sequence
  Primer
cttggcccgcatttacaagactatc

SEQ ID NO: 107 - DNA, 20 bp, Artificial Sequence
  Primer
cgtgcgtggagtaaaaaggt

SEQ ID NO: 108 - DNA, 20 bp, Artificial Sequence
  Primer
tgaacgcactctcactacgg

SEQ ID NO: 109 - DNA, 26 bp, Artificial Sequence
  Primer
gcccaatagaaagagaacaattgacc

SEQ ID NO: 110 - DNA, 23 bp, Artificial Sequence
  Primer
acacctccgcttacatcaacacc

SEQ ID NO: 111 - DNA, 20 bp, Artificial Sequence
  Primer
ggatcacgaggtcaggagat

SEQ ID NO: 112 - DNA, 19 bp, Artificial Sequence
  Primer
acggagtctcgctctgtcg

SEQ ID NO: 113 - DNA, 20 bp, Artificial Sequence
  Primer
gacctcgggatcatccttgc

SEQ ID NO: 114 - DNA, 17 bp, Artificial Sequence
  Primer
atggactggacctggag

SEQ ID NO: 115 - DNA, 22 bp, Artificial Sequence
  Primer
atggacacactttgctccacgc

SEQ ID NO: 116 - DNA, 21 bp, Artificial Sequence
  Primer
atgaaacacctgtggttcttc

SEQ ID NO: 117 - DNA, 21 bp, Artificial Sequence
  Primer
atgtctgtctccttcctcatc

SEQ ID NO: 118 - DNA, 20 bp, Artificial Sequence
  Primer
atggarttkggrctgagctg

SEQ ID NO: 119 - DNA, 18 bp, Artificial Sequence
  Primer
gtcaggatgtgggttttc

SEQ ID NO: 120 - DNA, 21 bp, Artificial Sequence
  Primer
ggaggtgccctgggctgtgtc

SEQ ID NO: 121 - DNA, 18 bp, Artificial Sequence
  Primer
gtgtctgggcacacactc

SEQ ID NO: 122 - DNA, 19 bp, Artificial Sequence
  Primer
ctcacactgacttcccctc

SEQ ID NO: 123 - DNA, 50 bp, Artificial Sequence
  Primer
ggaacagaccaccatggcccaggtbcagctggtgcagtctggggctgagg

SEQ ID NO: 124 - DNA, 42 bp, Artificial Sequence
  Primer
ggaacagaccaccatggcccaggtbcagctggtgcagtctgg

SEQ ID NO: 125 - DNA, 73 bp, Artificial Sequence
  Primer
gccgctggattgttattactcgcggcccagccggccatggcccaggtgcagctggtgcagtctggggctgagg

SEQ ID NO: 126 - DNA, 73 bp, Artificial Sequence
  Primer
gccgctggattgttattactcgcggcccagccggccatggcccaggtccagctcgtgcagtctggggctgagg

SEQ ID NO: 127 - DNA, 73 bp, Artificial Sequence
  Primer
gccgctggattgttattactcgcggcccagccggccatggcccaggttcagctggtgcagtctggagctgagg

SEQ ID NO: 128 - DNA, 73 bp, Artificial Sequence
  Primer
gccgctggattgttattactcgcggcccagccggccatggcccaggtccagctggtacagtctggggctgagg

SEQ ID NO: 129 - DNA, 65 bp, Artificial Sequence
  Primer
gccgctggattgttattactcgcggcccagccggccatggcccagrtcaccttgaaggagtctgg

SEQ ID NO: 130 - DNA, 42 bp, Artificial Sequence
  Primer
ggaacagaccaccatggcccagatcaccttgaaggagtctgg

SEQ ID NO: 131 - DNA, 48 bp, Artificial Sequence
  Primer
ggaacagaccaccatggccsaggtgcagctggtggagtctgggggagg

SEQ ID NO: 132 - DNA, 71 bp, Artificial Sequence
  Primer
gccgctggattgttattactcgcggcccagccggccatggccgaggtgcagctggtggagtctgggggagg

SEQ ID NO: 133 - DNA, 71 bp, Artificial Sequence
  Primer
gccgctggattgttattactcgcggcccagccggccatggccgaagtgcagctggtggagtctgggggagg

SEQ ID NO: 134 - DNA, 71 bp, Artificial Sequence
  Primer
gccgctggattgttattactcgcggcccagccggccatggcccaggtgcagctggtggagtctgggggagg

SEQ ID NO: 135 - DNA, 71 bp, Artificial Sequence
  Primer
gccgctggattgttattactcgcggcccagccggccatggccgaggtgcagctgttggagtctgggggagg

SEQ ID NO: 136 - DNA, 65 bp, Artificial Sequence
  Primer
gccgctggattgttattactcgcggcccagccggccatggcccaggtgcagctgcaggagtcggg

SEQ ID NO: 137 - DNA, 42 bp, Artificial Sequence
  Primer
ggaacagaccaccatggcccaggtgcagctgcaggagtcggg

SEQ ID NO: 138 - DNA, 66 bp, Artificial Sequence
  Primer
gccgctggattgttattactcgcggcccagccggccatggcccaggtgcagctacagcagtggggc

SEQ ID NO: 139 - DNA, 42 bp, Artificial Sequence
  Primer
ggaacagaccaccatggcccaggtacagctgcagcagtcagg

SEQ ID NO: 140 - DNA, 65 bp, Artificial Sequence
  Primer
gccgctggattgttattactcgcggcccagccggccatggcccaggtacagctgcagcagtcagg

SEQ ID NO: 141 - DNA, 34 bp, Artificial Sequence
  Primer
gctaccgccaccctcgagtgargagacrgtgacc

SEQ ID NO: 142 - DNA, 54 bp, Artificial Sequence
  Primer
ccgtggtgatggtggtgatggctaccgccaccctcgagtgargagacrgtgacc

SEQ ID NO: 143 - protein, 30 aa, Homo sapiens
  MISC_FEATURE: Hypervariable region
QVQLVESGGGLVQPGGSLRLSCAASGFTFS

SEQ ID NO: 144 - protein, 14 aa, Homo sapiens
  MISC_FEATURE: Hypervariable region
WVRQAPGKGLEWVA

SEQ ID NO: 145 - protein, 21 aa, Homo sapiens
  MISC_FEATURE: Hypervariable region
RFTISRDNAKNSLYLQMNSLR

SEQ ID NO: 146 - protein, 11 aa, Homo sapiens
  MISC_FEATURE: Hypervariable region
AEDTALYYCAR

SEQ ID NO: 147 - protein, 11 aa, Homo sapiens
  MISC_FEATURE: Hypervariable region
WGQGTTVTVSS